European Patent Specification EP 3 154 538 B1, published June 5, 2024. Title: Glycolic acid and/or D-lactic acid for the treatment of neurodegenerative diseases. Applicant: Max-Planck-Gesellschaft zur Förderung der Wissenschaften e.V. The sequence listing filed with the application follows.

SEQUENCE LISTING (9 sequences)

SEQ ID NO: 1 - DNA, 20 bp, Artificial Sequence
  source 1..20: /mol_type="unassigned DNA" /note="tm918_ext_fwd" /organism="Artificial Sequence"
cgacgagttgcgtatgagaa

SEQ ID NO: 2 - DNA, 20 bp, Artificial Sequence
  source 1..20: /mol_type="unassigned DNA" /note="tm918_ext_rev" /organism="Artificial Sequence"
cacaagtttttcggggagaa

SEQ ID NO: 3 - DNA, 20 bp, Artificial Sequence
  source 1..20: /mol_type="unassigned DNA" /note="tm918_int_fwd" /organism="Artificial Sequence"
tatgccggattagatggagc

SEQ ID NO: 4 - DNA, 20 bp, Artificial Sequence
  source 1..20: /mol_type="unassigned DNA" /note="tm951_ext_fwd" /organism="Artificial Sequence"
gatttcttcggcgtcttctg

SEQ ID NO: 5 - DNA, 20 bp, Artificial Sequence
  source 1..20: /mol_type="unassigned DNA" /note="tm951_ext_rev" /organism="Artificial Sequence"
cacatctcgggccactattt

SEQ ID NO: 6 - DNA, 20 bp, Artificial Sequence
  source 1..20: /mol_type="unassigned DNA" /note="tm951_int_fwd" /organism="Artificial Sequence"
aaaatgcaacgaccgacttc

SEQ ID NO: 7 - DNA, 20 bp, Artificial Sequence
  source 1..20: /mol_type="unassigned DNA" /note="tm1266_ext_fwd" /organism="Artificial Sequence"
tcctccgctcgctttttctc

SEQ ID NO: 8 - DNA, 20 bp, Artificial Sequence
  source 1..20: /mol_type="unassigned DNA" /note="tm1266_ext_rev" /organism="Artificial Sequence"
ttgcaagttgcttcgcatcc

SEQ ID NO: 9 - DNA, 20 bp, Artificial Sequence
  source 1..20: /mol_type="unassigned DNA" /note="tm1266_int_fwd" /organism="Artificial Sequence"
tcgaagctttggtcgtttcg